European Patent Application EP 4 653 020 A1, published November 26, 2025. Title: TYROSINASE-MEDIATED PROTEIN SITE-SPECIFIC CONJUGATION AND USE THEREOF. Applicant: SHANGHAI SHENGDI PHARMACEUTICAL CO., LTD. Application WO. The sequence listing filed with the application follows.

SEQUENCE LISTING (90 sequences)

SEQ ID NO: 1 - protein, 450 aa, synthetic construct
  source 1..450: note = Her wt HC
EVQLVESGGGLVQPGGSLRLSCAASGFNIKDTYIHWVRQAPGKGLEWVARIYPTNGYTRYADSVKGRFTISADTSKNTAYLQMNSLRAEDTAVYYCSRWGGDGFYAMDYWGQGTLVTVSSASTKGPSVFPLAPSSKSTSGGTAALGCLVKDYFPEPVTVSWNSGALTSGVHTFPAVLQSSGLYSLSSVVTVPSSSLGTQTYICNVNHKPSNTKVDKKVEPKSCDKTHTCPPCPAPELLGGPSVFLFPPKPKDTLMISRTPEVTCVVVDVSHEDPEVKFNWYVDGVEVHNAKTKPREEQYNSTYRVVSVLTVLHQDWLNGKEYKCKVSNKALPAPIEKTISKAKGQPREPQVYTLPPSREEMTKNQVSLTCLVKGFYPSDIAVEWESNGQPENNYKTTPPVLDSDGSFFLYSKLTVDKSRWQQGNVFSCSVMHEALHNHYTQKSLSLSPGK

SEQ ID NO: 2 - protein, 214 aa, synthetic construct
  source 1..214: note = Her wt LC
DIQMTQSPSSLSASVGDRVTITCRASQDVNTAVAWYQQKPGKAPKLLIYSASFLYSGVPSRFSGSRSGTDFTLTISSLQPEDFATYYCQQHYTTPPTFGQGTKVEIKRTVAAPSVFIFPPSDEQLKSGTASVVCLLNNFYPREAKVQWKVDNALQSGNSQESVTEQDSKDSTYSLSSTLTLSKADYEKHKVYACEVTHQGLSSPVTKSFNRGEC

SEQ ID NO: 3 - protein, 450 aa, synthetic construct
  source 1..450: note = Her H9 HC
EVQLVESGGGLVQPGGSLRLSCAASGFNIKDTYIHWVRQAPGKGLEWVARIYPTNGYTRYADSVKGRFTISADTSKNTAYLQMNSLRAEDTAVYYCSRWGGDGFYAMDYWGQGTLVTVSSASTKGPSVFPLAPSSKSYSGGTAALGCLVKDYFPEPVTVSWNSGALTSGVHTFPAVLQSSGLYSLSSVVTVPSSSLGTQTYICNVNHKPSNTKVDKKVEPKSCDKTHTCPPCPAPELLGGPSVFLFPPKPKDTLMISRTPEVTCVVVDVSHEDPEVKFNWYVDGVEVHNAKTKPREEQYNSTYRVVSVLTVLHQDWLNGKEYKCKVSNKALPAPIEKTISKAKGQPREPQVYTLPPSREEMTKNQVSLTCLVKGFYPSDIAVEWESNGQPENNYKTTPPVLDSDGSFFLYSKLTVDKSRWQQGNVFSCSVMHEALHNHYTQKSLSLSPGK

SEQ ID NO: 4 - protein, 450 aa, synthetic construct
  source 1..450: note = Her H10 HC
EVQLVESGGGLVQPGGSLRLSCAASGFNIKDTYIHWVRQAPGKGLEWVARIYPTNGYTRYADSVKGRFTISADTSKNTAYLQMNSLRAEDTAVYYCSRWGGDGFYAMDYWGQGTLVTVSSASTKGPSVFPLAPSSKSTSYGTAALGCLVKDYFPEPVTVSWNSGALTSGVHTFPAVLQSSGLYSLSSVVTVPSSSLGTQTYICNVNHKPSNTKVDKKVEPKSCDKTHTCPPCPAPELLGGPSVFLFPPKPKDTLMISRTPEVTCVVVDVSHEDPEVKFNWYVDGVEVHNAKTKPREEQYNSTYRVVSVLTVLHQDWLNGKEYKCKVSNKALPAPIEKTISKAKGQPREPQVYTLPPSREEMTKNQVSLTCLVKGFYPSDIAVEWESNGQPENNYKTTPPVLDSDGSFFLYSKLTVDKSRWQQGNVFSCSVMHEALHNHYTQKSLSLSPGK

SEQ ID NO: 5 - protein, 450 aa, synthetic construct
  source 1..450: note = Her H14 HC
EVQLVESGGGLVQPGGSLRLSCAASGFNIKDTYIHWVRQAPGKGLEWVARIYPTNGYTRYADSVKGRFTISADTSKNTAYLQMNSLRAEDTAVYYCSRWGGDGFYAMDYWGQGTLVTVSSASTKGPSVFPLAPSSKSTSGGTAALGCLVKDYFPEPVTVSWNSGALTSGVHTFPAVLQSSGLYSLSSVVTVPSSSLGTQYYICNVNHKPSNTKVDKKVEPKSCDKTHTCPPCPAPELLGGPSVFLFPPKPKDTLMISRTPEVTCVVVDVSHEDPEVKFNWYVDGVEVHNAKTKPREEQYNSTYRVVSVLTVLHQDWLNGKEYKCKVSNKALPAPIEKTISKAKGQPREPQVYTLPPSREEMTKNQVSLTCLVKGFYPSDIAVEWESNGQPENNYKTTPPVLDSDGSFFLYSKLTVDKSRWQQGNVFSCSVMHEALHNHYTQKSLSLSPGK

SEQ ID NO: 6 - protein, 450 aa, synthetic construct
  source 1..450: note = Her H19 HC
EVQLVESGGGLVQPGGSLRLSCAASGFNIKDTYIHWVRQAPGKGLEWVARIYPTNGYTRYADSVKGRFTISADTSKNTAYLQMNSLRAEDTAVYYCSRWGGDGFYAMDYWGQGTLVTVSSASTKGPSVFPLAPSSKSTSGGTAALGCLVKDYFPEPVTVSWNSGALTSGVHTFPAVLQSSGLYSLSSVVTVPSSSLGTQTYICNVNHKPSNTKVDKKVEPKSCDKYHTCPPCPAPELLGGPSVFLFPPKPKDTLMISRTPEVTCVVVDVSHEDPEVKFNWYVDGVEVHNAKTKPREEQYNSTYRVVSVLTVLHQDWLNGKEYKCKVSNKALPAPIEKTISKAKGQPREPQVYTLPPSREEMTKNQVSLTCLVKGFYPSDIAVEWESNGQPENNYKTTPPVLDSDGSFFLYSKLTVDKSRWQQGNVFSCSVMHEALHNHYTQKSLSLSPGK

SEQ ID NO: 7 - protein, 450 aa, synthetic construct
  source 1..450: note = Her H30 HC
EVQLVESGGGLVQPGGSLRLSCAASGFNIKDTYIHWVRQAPGKGLEWVARIYPTNGYTRYADSVKGRFTISADTSKNTAYLQMNSLRAEDTAVYYCSRWGGDGFYAMDYWGQGTLVTVSSASTKGPSVFPLAPSSKSTSGGTAALGCLVKDYFPEPVTVSWNSGALTSGVHTFPAVLQSSGLYSLSSVVTVPSSSLGTQTYICNVNHKPSNTKVDKKVEPKSCDKTHTCPPCPAPELLGGPSVFLFPPKPKDTLMISRTPEVTCVVVDVSHEDPEVKFNWYVDGVEVHNAKTKPREEQYNSTYRVVSVLTVLHQDWLNGKEYKCKVSNKALYAPIEKTISKAKGQPREPQVYTLPPSREEMTKNQVSLTCLVKGFYPSDIAVEWESNGQPENNYKTTPPVLDSDGSFFLYSKLTVDKSRWQQGNVFSCSVMHEALHNHYTQKSLSLSPGK

SEQ ID NO: 8 - protein, 450 aa, synthetic construct
  source 1..450: note = Her H33 HC
EVQLVESGGGLVQPGGSLRLSCAASGFNIKDTYIHWVRQAPGKGLEWVARIYPTNGYTRYADSVKGRFTISADTSKNTAYLQMNSLRAEDTAVYYCSRWGGDGFYAMDYWGQGTLVTVSSASTKGPSVFPLAPSSKSTSGGTAALGCLVKDYFPEPVTVSWNSGALTSGVHTFPAVLQSSGLYSLSSVVTVPSSSLGTQTYICNVNHKPSNTKVDKKVEPKSCDKTHTCPPCPAPELLGGPSVFLFPPKPKDTLMISRTPEVTCVVVDVSHEDPEVKFNWYVDGVEVHNAKTKPREEQYNSTYRVVSVLTVLHQDWLNGKEYKCKVSNKALPAPIEKTISKAKGYPREPQVYTLPPSREEMTKNQVSLTCLVKGFYPSDIAVEWESNGQPENNYKTTPPVLDSDGSFFLYSKLTVDKSRWQQGNVFSCSVMHEALHNHYTQKSLSLSPGK

SEQ ID NO: 9 - protein, 450 aa, synthetic construct
  source 1..450: note = Her H53 HC
EVQLVESGGGLVQPGGSLRLSCAASGFNIKDTYIHWVRQAPGKGLEWVARIYPTNGYTRYADSVKGRFTISADTSKNTAYLQMNSLRAEDTAVYYCSRWGGDGFYAMDYWGQGTLVTVSSASTKGPSVFPLAPSSKSTSGGTAALGCLVKDYFPEPVTVSWNSGALTSGVHTFPAVLQSSGLYSLSSVVTVPSSYLGTQTYICNVNHKPSNTKVDKKVEPKSCDKTHTCPPCPAPELLGGPSVFLFPPKPKDTLMISRTPEVTCVVVDVSHEDPEVKFNWYVDGVEVHNAKTKPREEQYNSTYRVVSVLTVLHQDWLNGKEYKCKVSNKALPAPIEKTISKAKGQPREPQVYTLPPSREEMTKNQVSLTCLVKGFYPSDIAVEWESNGQPENNYKTTPPVLDSDGSFFLYSKLTVDKSRWQQGNVFSCSVMHEALHNHYTQKSLSLSPGK

SEQ ID NO: 10 - protein, 450 aa, synthetic construct
  source 1..450: note = Her H26 HC
EVQLVESGGGLVQPGGSLRLSCAASGFNIKDTYIHWVRQAPGKGLEWVARIYPTNGYTRYADSVKGRFTISADTSKNTAYLQMNSLRAEDTAVYYCSRWGGDGFYAMDYWGQGTLVTVSSASTKGPSVFPLAPSSKSTSGGTAALGCLVKDYFPEPVTVSWNSGALTSGVHTFPAVLQSSGLYSLSSVVTVPSSSLGTQTYICNVNHKPSNTKVDKKVEPKSCDKTHTCPPCPAPELLGGPSVFLFPPKPKDTLMISRTPEVTCVVVDVSHEDPEVKFNWYVDGVEVHNAKTKPREEQFGYTFRVVSVLTVLHQDWLNGKEYKCKVSNKALPAPIEKTISKAKGQPREPQVYTLPPSREEMTKNQVSLTCLVKGFYPSDIAVEWESNGQPENNYKTTPPVLDSDGSFFLYSKLTVDKSRWQQGNVFSCSVMHEALHNHYTQKSLSLSPGK

SEQ ID NO: 11 - protein, 214 aa, synthetic construct
  source 1..214: note = Her L15 LC
DIQMTQSPSSLSASVGDRVTITCRASQDVNTAVAWYQQKPGKAPKLLIYSASFLYSGVPSRFSGSRSGTDFTLTISSLQPEDFATYYCQQHYTTPPTFGQGTKVEIKRTVAAPSVFIFPPSDEQLKSGTASVVCLLNNFYPREAKVQWKVDNALQSGNSQESVTEQDSKDSTYSLSSTLTLSKADYEKHKVYACEVTHQGLYSPVTKSFNRGEC

SEQ ID NO: 12 - protein, 445 aa, synthetic construct
  source 1..445: note = 0102 wt HC
EVQLVESGGGLVKPGGSLRLSCAASGFTFSTYAMSWVRQAPEKRLEWVATISDSDYYADNVKGRFTISRDNAKNSLYLQMNSLRAEDTAVYYCVRDDWDGDFDYWGQGTLVTVSSASTKGPSVFPLAPSSKSTSGGTAALGCLVKDYFPEPVTVSWNSGALTSGVHTFPAVLQSSGLYSLSSVVTVPSSSLGTQTYICNVNHKPSNTKVDKKVEPKSCDKTHTCPPCPAPELLGGPSVFLFPPKPKDTLMISRTPEVTCVVVDVSHEDPEVKFNWYVDGVEVHNAKTKPREEQYNSTYRVVSVLTVLHQDWLNGKEYKCKVSNKALPAPIEKTISKAKGQPREPQVYTLPPSREEMTKNQVSLTCLVKGFYPSDIAVEWESNGQPENNYKTTPPVLDSDGSFFLYSKLTVDKSRWQQGNVFSCSVMHEALHNHYTQKSLSLSPGK

SEQ ID NO: 13 - protein, 219 aa, synthetic construct
  source 1..219: note = 0102 wt LC
DVVMTQSPLSLPVTPGEPASISCKSTQSLLYSDGETYLNWLLQKPGQSPQRLIYLVSKLDSGVPDRFSGSGSGTDFTLKISRVEAEDVGVYYCWQGSHFPQTFGGGTKVEIKRTVAAPSVFIFPPSDEQLKSGTASVVCLLNNFYPREAKVQWKVDNALQSGNSQESVTEQDSKDSTYSLSSTLTLSKADYEKHKVYACEVTHQGLSSPVTKSFNRGEC

SEQ ID NO: 14 - protein, 445 aa, synthetic construct
  source 1..445: note = 0102 H9 HC
EVQLVESGGGLVKPGGSLRLSCAASGFTFSTYAMSWVRQAPEKRLEWVATISDSDYYADNVKGRFTISRDNAKNSLYLQMNSLRAEDTAVYYCVRDDWDGDFDYWGQGTLVTVSSASTKGPSVFPLAPSSKSYSGGTAALGCLVKDYFPEPVTVSWNSGALTSGVHTFPAVLQSSGLYSLSSVVTVPSSSLGTQTYICNVNHKPSNTKVDKKVEPKSCDKTHTCPPCPAPELLGGPSVFLFPPKPKDTLMISRTPEVTCVVVDVSHEDPEVKFNWYVDGVEVHNAKTKPREEQYNSTYRVVSVLTVLHQDWLNGKEYKCKVSNKALPAPIEKTISKAKGQPREPQVYTLPPSREEMTKNQVSLTCLVKGFYPSDIAVEWESNGQPENNYKTTPPVLDSDGSFFLYSKLTVDKSRWQQGNVFSCSVMHEALHNHYTQKSLSLSPGK

SEQ ID NO: 15 - protein, 445 aa, synthetic construct
  source 1..445: note = 0102 H10 HC
EVQLVESGGGLVKPGGSLRLSCAASGFTFSTYAMSWVRQAPEKRLEWVATISDSDYYADNVKGRFTISRDNAKNSLYLQMNSLRAEDTAVYYCVRDDWDGDFDYWGQGTLVTVSSASTKGPSVFPLAPSSKSTSYGTAALGCLVKDYFPEPVTVSWNSGALTSGVHTFPAVLQSSGLYSLSSVVTVPSSSLGTQTYICNVNHKPSNTKVDKKVEPKSCDKTHTCPPCPAPELLGGPSVFLFPPKPKDTLMISRTPEVTCVVVDVSHEDPEVKFNWYVDGVEVHNAKTKPREEQYNSTYRVVSVLTVLHQDWLNGKEYKCKVSNKALPAPIEKTISKAKGQPREPQVYTLPPSREEMTKNQVSLTCLVKGFYPSDIAVEWESNGQPENNYKTTPPVLDSDGSFFLYSKLTVDKSRWQQGNVFSCSVMHEALHNHYTQKSLSLSPGK

SEQ ID NO: 16 - protein, 445 aa, synthetic construct
  source 1..445: note = 0102 H19 HC
EVQLVESGGGLVKPGGSLRLSCAASGFTFSTYAMSWVRQAPEKRLEWVATISDSDYYADNVKGRFTISRDNAKNSLYLQMNSLRAEDTAVYYCVRDDWDGDFDYWGQGTLVTVSSASTKGPSVFPLAPSSKSTSGGTAALGCLVKDYFPEPVTVSWNSGALTSGVHTFPAVLQSSGLYSLSSVVTVPSSSLGTQTYICNVNHKPSNTKVDKKVEPKSCDKYHTCPPCPAPELLGGPSVFLFPPKPKDTLMISRTPEVTCVVVDVSHEDPEVKFNWYVDGVEVHNAKTKPREEQYNSTYRVVSVLTVLHQDWLNGKEYKCKVSNKALPAPIEKTISKAKGQPREPQVYTLPPSREEMTKNQVSLTCLVKGFYPSDIAVEWESNGQPENNYKTTPPVLDSDGSFFLYSKLTVDKSRWQQGNVFSCSVMHEALHNHYTQKSLSLSPGK

SEQ ID NO: 17 - protein, 445 aa, synthetic construct
  source 1..445: note = 0102 H30 HC
EVQLVESGGGLVKPGGSLRLSCAASGFTFSTYAMSWVRQAPEKRLEWVATISDSDYYADNVKGRFTISRDNAKNSLYLQMNSLRAEDTAVYYCVRDDWDGDFDYWGQGTLVTVSSASTKGPSVFPLAPSSKSTSGGTAALGCLVKDYFPEPVTVSWNSGALTSGVHTFPAVLQSSGLYSLSSVVTVPSSSLGTQTYICNVNHKPSNTKVDKKVEPKSCDKTHTCPPCPAPELLGGPSVFLFPPKPKDTLMISRTPEVTCVVVDVSHEDPEVKFNWYVDGVEVHNAKTKPREEQYNSTYRVVSVLTVLHQDWLNGKEYKCKVSNKALYAPIEKTISKAKGQPREPQVYTLPPSREEMTKNQVSLTCLVKGFYPSDIAVEWESNGQPENNYKTTPPVLDSDGSFFLYSKLTVDKSRWQQGNVFSCSVMHEALHNHYTQKSLSLSPGK

SEQ ID NO: 18 - protein, 445 aa, synthetic construct
  source 1..445: note = 0102 H53 HC
EVQLVESGGGLVKPGGSLRLSCAASGFTFSTYAMSWVRQAPEKRLEWVATISDSDYYADNVKGRFTISRDNAKNSLYLQMNSLRAEDTAVYYCVRDDWDGDFDYWGQGTLVTVSSASTKGPSVFPLAPSSKSTSGGTAALGCLVKDYFPEPVTVSWNSGALTSGVHTFPAVLQSSGLYSLSSVVTVPSSYLGTQTYICNVNHKPSNTKVDKKVEPKSCDKTHTCPPCPAPELLGGPSVFLFPPKPKDTLMISRTPEVTCVVVDVSHEDPEVKFNWYVDGVEVHNAKTKPREEQYNSTYRVVSVLTVLHQDWLNGKEYKCKVSNKALPAPIEKTISKAKGQPREPQVYTLPPSREEMTKNQVSLTCLVKGFYPSDIAVEWESNGQPENNYKTTPPVLDSDGSFFLYSKLTVDKSRWQQGNVFSCSVMHEALHNHYTQKSLSLSPGK

SEQ ID NO: 19 - protein, 445 aa, synthetic construct
  source 1..445: note = 0102 H26 HC
EVQLVESGGGLVKPGGSLRLSCAASGFTFSTYAMSWVRQAPEKRLEWVATISDSDYYADNVKGRFTISRDNAKNSLYLQMNSLRAEDTAVYYCVRDDWDGDFDYWGQGTLVTVSSASTKGPSVFPLAPSSKSTSGGTAALGCLVKDYFPEPVTVSWNSGALTSGVHTFPAVLQSSGLYSLSSVVTVPSSSLGTQTYICNVNHKPSNTKVDKKVEPKSCDKTHTCPPCPAPELLGGPSVFLFPPKPKDTLMISRTPEVTCVVVDVSHEDPEVKFNWYVDGVEVHNAKTKPREEQFGYTFRVVSVLTVLHQDWLNGKEYKCKVSNKALPAPIEKTISKAKGQPREPQVYTLPPSREEMTKNQVSLTCLVKGFYPSDIAVEWESNGQPENNYKTTPPVLDSDGSFFLYSKLTVDKSRWQQGNVFSCSVMHEALHNHYTQKSLSLSPGK

SEQ ID NO: 20 - protein, 219 aa, synthetic construct
  source 1..219: note = 0102 L15 LC
DVVMTQSPLSLPVTPGEPASISCKSTQSLLYSDGETYLNWLLQKPGQSPQRLIYLVSKLDSGVPDRFSGSGSGTDFTLKISRVEAEDVGVYYCWQGSHFPQTFGGGTKVEIKRTVAAPSVFIFPPSDEQLKSGTASVVCLLNNFYPREAKVQWKVDNALQSGNSQESVTEQDSKDSTYSLSSTLTLSKADYEKHKVYACEVTHQGLYSPVTKSFNRGEC

SEQ ID NO: 21 - protein, 305 aa, synthetic construct
  source 1..305: note = megaTYR
MSNKYRVRKNVLHLTDTEKRDFVRTVLILKEKGIYDRYIAWHGAAGKFHTPPGSDRNAAHMSSAFLPWHREYLLRFERDLQSINPEVTLPYWEWETDAQMQDPSQSQIWSADFMGGNGNPIKDFIVDTGPFAAGRWTTIDEQGNPSGGLKRNFGATKEAPTLPTRDDVLNALKITQYDTPPWDMTSQNSFRNQLEGFINGPQLHNRVHRWVGGQMGVVPTAPNDPVFFLHHANVDRIWAVWQIIHRNQNYQPMKNGPFGQNFRDPMYPWNTTPEDVMNHRKLGYVYDIELRKSKRSSLEHHHHHH

SEQ ID NO: 22 - protein, 342 aa, synthetic construct
  source 1..342: note = VsTYR core
MAKYHRLNLQNPAAAPFLESYKKAITVMLQLPPSDARNWYRNAFIHTLDCPHGNWWFVVWHRGYTGWFERTVRELSGDPNFAFPYWDWTALPQVPDSFFNGVLDPNNPAFIASYNEFYSQLSNPMSALWNSFSTAQLQQMRNRGFQSVNDVWQAVRDSPMFFPRGRARTLTRQNPGFDATTRRAVSIGTIRNALAPTDFITFGSGKTANHSESATQGILESQPHNNVHNNIGGFMQDLLSPTDPVFFAHHSNIDRLWDVWTRKQQRLGLPTLPTGANLPLWANEPFLFFIGPDGKPVAKNKAGDYATIGDFEYNYEPGSGEAVIPAASRPGEMNNKHHHHHH

SEQ ID NO: 23 - protein, 364 aa, synthetic construct
  source 1..364: note = VsTYR sp
MRGSHHHHHHGMASMTGGQQMGRDLYDDDDKDPSSRSAAGTMAKYHRLNLQNPAAAPFLESYKKAITVMLQLPPSDARNWYRNAFIHTLDCPHGNWWFVVWHRGYTGWFERTVRELSGDPNFAFPYWDWTALPQVPDSFFNGVLDPNNPAFIASYNEFYSQLSNPMSALWNSFSTAQLQQMRNRGFQSVNDVWQAVRDSPMFFPRGRARTLTRQNPGFDATTRRAVSIGTIRNALAPTDFITFGSGKTANHSESATQGILESQPHNNVHNNIGGFMQDLLSPTDPVFFAHHSNIDRLWDVWTRKQQRLGLPTLPTGANLPLWANEPFLFFIGPDGKPVAKNKAGDYATIGDFEYNYEPGSGEAV

SEQ ID NO: 24 - protein, 450 aa, synthetic construct
  source 1..450: note = Her HH3 HC
EVQLVESGGGLVQPGGSLRLSCAASGFNIKDTYIHWVRQAPGKGLEWVARIYPTNGYTRYADSVKGRFTISADTSKNTAYLQMNSLRAEDTAVYYCSRWGGDGFYAMDYWGQGTLVTVSSASTKGPSVFPLAPSSKSYSGGTAALGCLVKDYFPEPVTVSWNSGALTSGVHTFPAVLQSSGLYSLSSVVTVPSSSLGTQTYICNVNHKPSNTKVDKKVEPKSCDKYHTCPPCPAPELLGGPSVFLFPPKPKDTLMISRTPEVTCVVVDVSHEDPEVKFNWYVDGVEVHNAKTKPREEQYNSTYRVVSVLTVLHQDWLNGKEYKCKVSNKALYAPIEKTISKAKGQPREPQVYTLPPSREEMTKNQVSLTCLVKGFYPSDIAVEWESNGQPENNYKTTPPVLDSDGSFFLYSKLTVDKSRWQQGNVFSCSVMHEALHNHYTQKSLSLSPGK

SEQ ID NO: 25 - protein, 450 aa, synthetic construct
  source 1..450: note = Her HH4 HC
EVQLVESGGGLVQPGGSLRLSCAASGFNIKDTYIHWVRQAPGKGLEWVARIYPTNGYTRYADSVKGRFTISADTSKNTAYLQMNSLRAEDTAVYYCSRWGGDGFYAMDYWGQGTLVTVSSASTKGPSVFPLAPSSKSYSGGTAALGCLVKDYFPEPVTVSWNSGALTSGVHTFPAVLQSSGLYSLSSVVTVPSSYLGTQTYICNVNHKPSNTKVDKKVEPKSCDKYHTCPPCPAPELLGGPSVFLFPPKPKDTLMISRTPEVTCVVVDVSHEDPEVKFNWYVDGVEVHNAKTKPREEQYNSTYRVVSVLTVLHQDWLNGKEYKCKVSNKALYAPIEKTISKAKGQPREPQVYTLPPSREEMTKNQVSLTCLVKGFYPSDIAVEWESNGQPENNYKTTPPVLDSDGSFFLYSKLTVDKSRWQQGNVFSCSVMHEALHNHYTQKSLSLSPGK

SEQ ID NO: 26 - protein, 450 aa, synthetic construct
  source 1..450: note = Her HH8 HC
EVQLVESGGGLVQPGGSLRLSCAASGFNIKDTYIHWVRQAPGKGLEWVARIYPTNGYTRYADSVKGRFTISADTSKNTAYLQMNSLRAEDTAVYYCSRWGGDGFYAMDYWGQGTLVTVSSASTKGPSVFPLAPSSKSYSGGTAALGCLVKDYFPEPVTVSWNSGALTSGVHTFPAVLQSSGLYSLSSVVTVPSSSLGTQTYICNVNHKPSNTKVDKKVEPKSCDKTHTCPPCPAPELLGGPSVFLFPPKPKDTLMISRTPEVTCVVVDVSHEDPEVKFNWYVDGVEVHNAKTKPREEQYNSTYRVVSVLTVLHQDWLNGKEYKCKVSNKALYAPIEKTISKAKGQPREPQVYTLPPSREEMTKNQVSLTCLVKGFYPSDIAVEWESNGQPENNYKTTPPVLDSDGSFFLYSKLTVDKSRWQQGNVFSCSVMHEALHNHYTQKSLSLSPGK

SEQ ID NO: 27 - protein, 450 aa, synthetic construct
  source 1..450: note = Her HH9 HC
EVQLVESGGGLVQPGGSLRLSCAASGFNIKDTYIHWVRQAPGKGLEWVARIYPTNGYTRYADSVKGRFTISADTSKNTAYLQMNSLRAEDTAVYYCSRWGGDGFYAMDYWGQGTLVTVSSASTKGPSVFPLAPSSKSTSGGTAALGCLVKDYFPEPVTVSWNSGALTSGVHTFPAVLQSSGLYSLSSVVTVPSSSLGTQTYICNVNHKPSNTKVDKKVEPKSCDKYHTCPPCPAPELLGGPSVFLFPPKPKDTLMISRTPEVTCVVVDVSHEDPEVKFNWYVDGVEVHNAKTKPREEQYNSTYRVVSVLTVLHQDWLNGKEYKCKVSNKALYAPIEKTISKAKGQPREPQVYTLPPSREEMTKNQVSLTCLVKGFYPSDIAVEWESNGQPENNYKTTPPVLDSDGSFFLYSKLTVDKSRWQQGNVFSCSVMHEALHNHYTQKSLSLSPGK

SEQ ID NO: 28 - protein, 441 aa, synthetic construct
  source 1..441: note = 0102 H73 HC
EVQLVESGGGLVKPGGSLRLSCAASGFTFSTYAMSWVRQAPEKRLEWVATISDSDYYADNVKGRFTISRDNAKNSLYLQMNSLRAEDTAVYYCVRDDWDGDFDYWGQGTLVTVSSASTKGPSVFPLAPCSRSTSESTAALGCLVKDYFPEPVTVSWNSGALTSGVHTFPAVLQSSGLYSLSSVVTVPSSNFGTQTYTCNVDHKPSNTKVDKTVERKCCVECPPCPAPPVAGPSVFLFPPKPKDTLMISRTPEVTCVVVDVSHEDPEVQFNWYVDGVEVHNAKTKPREEQFNSTFRVVSVLTVVHQDWLNGKEYKCKVSNKGLPAPIEKTISKTKGQPREPQVYTLPPSREEMTKNQVSLTCLVKGFYPSDISVEWESNGQPENNYKTTPPMLDSDGSFFLYSKLTVDKSRWQQGNVFSCSVMHEALHNHYTQKSLSLSPGK

SEQ ID NO: 29 - protein, 492 aa, synthetic construct
  source 1..492: note = 0102 H74 HC
EVQLVESGGGLVKPGGSLRLSCAASGFTFSTYAMSWVRQAPEKRLEWVATISDSDYYADNVKGRFTISRDNAKNSLYLQMNSLRAEDTAVYYCVRDDWDGDFDYWGQGTLVTVSSASTKGPSVFPLAPCSRSTSGGTAALGCLVKDYFPEPVTVSWNSGALTSGVHTFPAVLQSSGLYSLSSVVTVPSSSLGTQTYTCNVNHKPSNTKVDKRVELKTPLGDTTHTCPRCPEPKSCDTPPPCPRCPEPKSCDTPPPCPRCPEPKSCDTPPPCPRCPAPELLGGPSVFLFPPKPKDTLMISRTPEVTCVVVDVSHEDPEVQFKWYVDGVEVHNAKTKPREEQFNSTFRVVSVLTVLHQDWLNGKEYKCKVSNKALPAPIEKTISKTKGQPREPQVYTLPPSREEMTKNQVSLTCLVKGFYPSDIAVEWESSGQPENNYNTTPPMLDSDGSFFLYSKLTVDKSRWQQGNIFSCSVMHEALHNRFTQKSLSLSPGK

SEQ ID NO: 30 - protein, 442 aa, synthetic construct
  source 1..442: note = 0102 H40 HC
EVQLVESGGGLVKPGGSLRLSCAASGFTFSTYAMSWVRQAPEKRLEWVATISDSDYYADNVKGRFTISRDNAKNSLYLQMNSLRAEDTAVYYCVRDDWDGDFDYWGQGTLVTVSSASTKGPSVFPLAPCSRSTSESTAALGCLVKDYFPEPVTVSWNSGALTSGVHTFPAVLQSSGLYSLSSVVTVPSSSLGTKTYTCNVDHKPSNTKVDKRVESKYGPPCPPCPAPEFLGGPSVFLFPPKPKDTLMISRTPEVTCVVVDVSQEDPEVQFNWYVDGVEVHNAKTKPREEQFNSTYRVVSVLTVLHQDWLNGKEYKCKVSNKGLPSSIEKTISKAKGQPREPQVYTLPPSQEEMTKNQVSLTCLVKGFYPSDIAVEWESNGQPENNYKTTPPVLDSDGSFFLYSRLTVDKSRWQEGNVFSCSVMHEALHNHYTQKSLSLSLGK

SEQ ID NO: 31 - protein, 441 aa, synthetic construct
  source 1..441: note = 0102 H75 HC
EVQLVESGGGLVKPGGSLRLSCAASGFTFSTYAMSWVRQAPEKRLEWVATISDSDYYADNVKGRFTISRDNAKNSLYLQMNSLRAEDTAVYYCVRDDWDGDFDYWGQGTLVTVSSASTKGPSVFPLAPCSRSYSESTAALGCLVKDYFPEPVTVSWNSGALTSGVHTFPAVLQSSGLYSLSSVVTVPSSNFGTQTYTCNVDHKPSNTKVDKTVERKCCVECPPCPAPPVAGPSVFLFPPKPKDTLMISRTPEVTCVVVDVSHEDPEVQFNWYVDGVEVHNAKTKPREEQFNSTFRVVSVLTVVHQDWLNGKEYKCKVSNKGLPAPIEKTISKTKGQPREPQVYTLPPSREEMTKNQVSLTCLVKGFYPSDISVEWESNGQPENNYKTTPPMLDSDGSFFLYSKLTVDKSRWQQGNVFSCSVMHEALHNHYTQKSLSLSPGK

SEQ ID NO: 32 - protein, 441 aa, synthetic construct
  source 1..441: note = 0102 H76 HC
EVQLVESGGGLVKPGGSLRLSCAASGFTFSTYAMSWVRQAPEKRLEWVATISDSDYYADNVKGRFTISRDNAKNSLYLQMNSLRAEDTAVYYCVRDDWDGDFDYWGQGTLVTVSSASTKGPSVFPLAPCSRSTSESTAALGCLVKDYFPEPVTVSWNSGALTSGVHTFPAVLQSSGLYSLSSVVTVPSSYFGTQTYTCNVDHKPSNTKVDKTVERKCCVECPPCPAPPVAGPSVFLFPPKPKDTLMISRTPEVTCVVVDVSHEDPEVQFNWYVDGVEVHNAKTKPREEQFNSTFRVVSVLTVVHQDWLNGKEYKCKVSNKGLPAPIEKTISKTKGQPREPQVYTLPPSREEMTKNQVSLTCLVKGFYPSDISVEWESNGQPENNYKTTPPMLDSDGSFFLYSKLTVDKSRWQQGNVFSCSVMHEALHNHYTQKSLSLSPGK

SEQ ID NO: 33 - protein, 492 aa, synthetic construct
  source 1..492: note = 0102 H77 HC
EVQLVESGGGLVKPGGSLRLSCAASGFTFSTYAMSWVRQAPEKRLEWVATISDSDYYADNVKGRFTISRDNAKNSLYLQMNSLRAEDTAVYYCVRDDWDGDFDYWGQGTLVTVSSASTKGPSVFPLAPCSRSTSGGTAALGCLVKDYFPEPVTVSWNSGALTSGVHTFPAVLQSSGLYSLSSVVTVPSSSLGTQTYTCNVNHKPSNTKVDKRVELKTPLGDTTHTCPRCPEPKSCDTPPPCPRCPEPKSCDTPPPCPRCPEPKSCDTPPPCPRCPAPELLGGPSVFLFPPKPKDTLMISRTPEVTCVVVDVSHEDPEVQFKWYVDGVEVHNAKTKPREEQFNSTFRVVSVLTVLHQDWLNGKEYKCKVSNKALYAPIEKTISKTKGQPREPQVYTLPPSREEMTKNQVSLTCLVKGFYPSDIAVEWESSGQPENNYNTTPPMLDSDGSFFLYSKLTVDKSRWQQGNIFSCSVMHEALHNRFTQKSLSLSPGK

SEQ ID NO: 34 - protein, 442 aa, synthetic construct
  source 1..442: note = 0102 H78 HC
EVQLVESGGGLVKPGGSLRLSCAASGFTFSTYAMSWVRQAPEKRLEWVATISDSDYYADNVKGRFTISRDNAKNSLYLQMNSLRAEDTAVYYCVRDDWDGDFDYWGQGTLVTVSSASTKGPSVFPLAPCSRSYSESTAALGCLVKDYFPEPVTVSWNSGALTSGVHTFPAVLQSSGLYSLSSVVTVPSSSLGTKTYTCNVDHKPSNTKVDKRVESKYGPPCPPCPAPEFLGGPSVFLFPPKPKDTLMISRTPEVTCVVVDVSQEDPEVQFNWYVDGVEVHNAKTKPREEQFNSTYRVVSVLTVLHQDWLNGKEYKCKVSNKGLPSSIEKTISKAKGQPREPQVYTLPPSQEEMTKNQVSLTCLVKGFYPSDIAVEWESNGQPENNYKTTPPVLDSDGSFFLYSRLTVDKSRWQEGNVFSCSVMHEALHNHYTQKSLSLSLGK

SEQ ID NO: 35 - protein, 442 aa, synthetic construct
  source 1..442: note = 0102 H79 HC
EVQLVESGGGLVKPGGSLRLSCAASGFTFSTYAMSWVRQAPEKRLEWVATISDSDYYADNVKGRFTISRDNAKNSLYLQMNSLRAEDTAVYYCVRDDWDGDFDYWGQGTLVTVSSASTKGPSVFPLAPCSRSTSESTAALGCLVKDYFPEPVTVSWNSGALTSGVHTFPAVLQSSGLYSLSSVVTVPSSSLGTKTYTCNVDHKPSNTKVDKRVESKYGPPCPPCPAPEFLGGPSVFLFPPKPKDTLMISRTPEVTCVVVDVSQEDPEVQFNWYVDGVEVHNAKTKPREEQFNSTYRVVSVLTVLHQDWLNGKEYKCKVSNKGLYSSIEKTISKAKGQPREPQVYTLPPSQEEMTKNQVSLTCLVKGFYPSDIAVEWESNGQPENNYKTTPPVLDSDGSFFLYSRLTVDKSRWQEGNVFSCSVMHEALHNHYTQKSLSLSLGK

SEQ ID NO: 36 - protein, 450 aa, synthetic construct
  source 1..450: note = c-met H10 HC
QVQLVESGGGVVQPGRSLRLSCAASGFSLSNYGVHWVRQAPGKGLEWLAVIWSGGSTNYAAAFVSRLTISKDNSKNTVYLQMNSLRAEDTAVYYCARNHDNPYNYAMDYWGQGTTVTVSSASTKGPSVFPLAPSSKSTSYGTAALGCLVKDYFPEPVTVSWNSGALTSGVHTFPAVLQSSGLYSLSSVVTVPSSSLGTQTYICNVNHKPSNTKVDKKVEPKSCDKTHTCPPCPAPELLGGPSVFLFPPKPKDTLMISRTPEVTCVVVDVSHEDPEVKFNWYVDGVEVHNAKTKPREEQYNSTYRVVSVLTVLHQDWLNGKEYKCKVSNKALPAPIEKTISKAKGQPREPQVYTLPPSREEMTKNQVSLTCLVKGFYPSDIAVEWESNGQPENNYKTTPPVLDSDGSFFLYSKLTVDKSRWQQGNVFSCSVMHEALHNHYTQKSLSLSPGK

SEQ ID NO: 37 - protein, 218 aa, synthetic construct
  source 1..218: note = c-met H10 LC
DIVLTQSPDSLAVSLGERATINCRADKSVSTSTYNYLHWYQQKPGQPPKLLIYLASNLASGVPDRFSGSGSGTDFTLTISSLQAEDVAVYYCQHSRDLPPTFGQGTKLEIKRTVAAPSVFIFPPSDEQLKSGTASVVCLLNNFYPREAKVQWKVDNALQSGNSQESVTEQDSKDSTYSLSSTLTLSKADYEKHKVYACEVTHQGLSSPVTKSFNRGEC

SEQ ID NO: 38 - protein, 450 aa, synthetic construct
  source 1..450: note = c-met L15 HC
QVQLVESGGGVVQPGRSLRLSCAASGFSLSNYGVHWVRQAPGKGLEWLAVIWSGGSTNYAAAFVSRLTISKDNSKNTVYLQMNSLRAEDTAVYYCARNHDNPYNYAMDYWGQGTTVTVSSASTKGPSVFPLAPSSKSTSGGTAALGCLVKDYFPEPVTVSWNSGALTSGVHTFPAVLQSSGLYSLSSVVTVPSSSLGTQTYICNVNHKPSNTKVDKKVEPKSCDKTHTCPPCPAPELLGGPSVFLFPPKPKDTLMISRTPEVTCVVVDVSHEDPEVKFNWYVDGVEVHNAKTKPREEQYNSTYRVVSVLTVLHQDWLNGKEYKCKVSNKALPAPIEKTISKAKGQPREPQVYTLPPSREEMTKNQVSLTCLVKGFYPSDIAVEWESNGQPENNYKTTPPVLDSDGSFFLYSKLTVDKSRWQQGNVFSCSVMHEALHNHYTQKSLSLSPGK

SEQ ID NO: 39 - protein, 218 aa, synthetic construct
  source 1..218: note = c-met L15 LC
DIVLTQSPDSLAVSLGERATINCRADKSVSTSTYNYLHWYQQKPGQPPKLLIYLASNLASGVPDRFSGSGSGTDFTLTISSLQAEDVAVYYCQHSRDLPPTFGQGTKLEIKRTVAAPSVFIFPPSDEQLKSGTASVVCLLNNFYPREAKVQWKVDNALQSGNSQESVTEQDSKDSTYSLSSTLTLSKADYEKHKVYACEVTHQGLYSPVTKSFNRGEC

SEQ ID NO: 40 - protein, 437 aa, synthetic construct
  source 1..437: note = ADA mut HC
DIQMTQSPSSLSASVGDRVTITCRASQGIRNYLAWYQQKPGKAPKLLIYAASTLQSGVPSRFSGSGSGTDFTLTISSLQPEDVATYYCQRYNRAPYTFGQGTKVEIKASTKGPSVFPLAPSSKSTSGGTAALGCLVKDYFPEPVTVSWNSGALTSGVHTFPAVLQSSGLYSLSSVVTVPSSSLGTQTYICNVNHKPSNTKVDKKVEPKSCDKTHTCPPCPAPELLGGPSVFLFPPKPKDTLMISRTPEVTCVVVDVSHEDPEVKFNWYVDGVEVHNAKTKPREEQYNSTYRVVSVLTVLHQDWLNGKEYKCKVSNKALYAPIEKTISKAKGQPREPQVYTLPPSREEMTKNQVSLTCLVKGFYPSDIAVEWESNGQPENNYKTTPPVLDSDGSFFLYSKLTVDKSRWQQGNVFSCSVMHEALHNHYTQKSLSLSPGK

SEQ ID NO: 41 - protein, 219 aa, synthetic construct
  source 1..219: note = ADA mut LC
DAVMTQTPLSLSVTPGQPASISCRSSQSLERSTGNTFLNWYLQKPGQSPQLLIYRVSTRFSGVPDRFSGSGSGTDFTLKISRVEAEDVGVYYCLQLTHVPLTFGGGTKVEIKRTVAAPSVFIFPPSDEQLKSGTASVVCLLNNFYPREAKVQWKVDNALQSGNSQESVTEQDSKDSTYSLSSTLTLSKADYEKHKVYACEVTHQGLYSPVTKSFNRGEC

SEQ ID NO: 42 - protein, 451 aa, synthetic construct
  source 1..451: note = trop2 mut HC
EVQLVESGGGLVQPGRSLRLSCAASGFTFDDYAMHWVRQAPGKGLEWVSAITWNSGHIDYADSVEGRFTISRDNAKNSLYLQMNSLRAEDTAVYYCAKVSYLSTASSLDYWGQGTLVTVSSASTKGPSVFPLAPSSKSTSYGTAALGCLVKDYFPEPVTVSWNSGALTSGVHTFPAVLQSSGLYSLSSVVTVPSSSLGTQTYICNVNHKPSNTKVDKKVEPKSCDKTHTCPPCPAPELLGGPSVFLFPPKPKDTLMISRTPEVTCVVVDVSHEDPEVKFNWYVDGVEVHNAKTKPREEQYNSTYRVVSVLTVLHQDWLNGKEYKCKVSNKALPAPIEKTISKAKGQPREPQVYTLPPSREEMTKNQVSLTCLVKGFYPSDIAVEWESNGQPENNYKTTPPVLDSDGSFFLYSKLTVDKSRWQQGNVFSCSVMHEALHNHYTQKSLSLSPGK

SEQ ID NO: 43 - protein, 214 aa, synthetic construct
  source 1..214: note = trop2 mut LC
DIQMTQSPSSLSASVGDRVTITCRASQGIRNYLAWYQQKPGKAPKLLIYAASTLQSGVPSRFSGSGSGTDFTLTISSLQPEDVATYYCQRYNRAPYTFGQGTKVEIKRTVAAPSVFIFPPSDEQLKSGTASVVCLLNNFYPREAKVQWKVDNALQSGNSQESVTEQDSKDSTYSLSSTLTLSKADYEKHKVYACEVTHQGLYSPVTKSFNRGEC

SEQ ID NO: 44 - protein, 451 aa, synthetic construct
  source 1..451: note = ADC-2 HC
EVQLVESGGGLVQPGRSLRLSCAASGFTFDDYAMHWVRQAPGKGLEWVSAITWNSGHIDYADSVEGRFTISRDNAKNSLYLQMNSLRAEDTAVYYCAKVSYLSTASSLDYWGQGTLVTVSSASTKGPSVFPLAPSSKSTSGGTAALGCLVKDYFPEPVTVSWNSGALTSGVHTFPAVLQSSGLYSLSSVVTVPSSSLGTQTYICNVNHKPSNTKVDKKVEPKSCDKTHTCPPCPAPELLGGPSVFLFPPKPKDTLMISRTPEVTCVVVDVSHEDPEVKFNWYVDGVEVHNAKTKPREEQYNSTYRVVSVLTVLHQDWLNGKEYKCKVSNKALYAPIEKTISKAKGQPREPQVYTLPPSREEMTKNQVSLTCLVKGFYPSDIAVEWESNGQPENNYKTTPPVLDSDGSFFLYSKLTVDKSRWQQGNVFSCSVMHEALHNHYTQKSLSLSPGK

SEQ ID NO: 45 - protein, 214 aa, synthetic construct
  source 1..214: note = ADC-2 LC
DIQMTQSPSSLSASVGDRVTITCRASQGIRNYLAWYQQKPGKAPKLLIYAASTLQSGVPSRFSGSGSGTDFTLTISSLQPEDVATYYCQRYNRAPYTFGQGTKVEIKRTVAAPSVFIFPPSDEQLKSGTASVVCLLNNFYPREAKVQWKVDNALQSGNSQESVTEQDSKDSTYSLSSTLTLSKADYEKHKVYACEVTHQGLSSPVTKSFNRGEC

SEQ ID NO: 46 - protein, 98 aa, synthetic construct
  source 1..98: note = CH1
ASTKGPSVFPLAPSSKSTSGGTAALGCLVKDYFPEPVTVSWNSGALTSGVHTFPAVLQSSGLYSLSSVVTVPSSSLGTQTYICNVNHKPSNTKVDKKV

SEQ ID NO: 47 - protein, 15 aa, synthetic construct
  source 1..15: note = hinge
EPKSCDKTHTCPPCP

SEQ ID NO: 48 - protein, 110 aa, synthetic construct
  source 1..110: note = CH2
APELLGGPSVFLFPPKPKDTLMISRTPEVTCVVVDVSHEDPEVKFNWYVDGVEVHNAKTKPREEQYNSTYRVVSVLTVLHQDWLNGKEYKCKVSNKALPAPIEKTISKAK

SEQ ID NO: 49 - protein, 107 aa, synthetic construct
  source 1..107: note = CH3
GQPREPQVYTLPPSREEMTKNQVSLTCLVKGFYPSDIAVEWESNGQPENNYKTTPPVLDSDGSFFLYSKLTVDKSRWQQGNVFSCSVMHEALHNHYTQKSLSLSPGK

SEQ ID NO: 50 - protein, 107 aa, synthetic construct [sequence omitted]

SEQ ID NO: 51 - protein, 5 aa, synthetic construct
  source 1..5: note = CDR
DTYIH

SEQ ID NO: 52 - protein, 17 aa, synthetic construct
  source 1..17: note = CDR
RIYPTNGYTRYADSVKG

SEQ ID NO: 53 - protein, 11 aa, synthetic construct
  source 1..11: note = CDR
WGGDGFYAMDY

SEQ ID NO: 54 - protein, 11 aa, synthetic construct
  source 1..11: note = CDR
RASQDVNTAVA

SEQ ID NO: 55 - protein, 7 aa, synthetic construct
  source 1..7: note = CDR
SASFLYS

SEQ ID NO: 56 - protein, 9 aa, synthetic construct
  source 1..9: note = CDR
QQHYTTPPT

SEQ ID NO: 57 - protein, 120 aa, synthetic construct [sequence omitted]

SEQ ID NO: 58 - protein, 107 aa, synthetic construct [sequence omitted]

SEQ ID NO: 59 - protein, 5 aa, synthetic construct
  source 1..5: note = CDR
TYAMS

SEQ ID NO: 60 - protein, 14 aa, synthetic construct
  source 1..14: note = CDR
TISDSDYYADNVKG

SEQ ID NO: 61 - protein, 9 aa, synthetic construct
  source 1..9: note = CDR
DDWDGDFDY

SEQ ID NO: 62 - protein, 16 aa, synthetic construct
  source 1..16: note = CDR
KSTQSLLYSDGETYLN

SEQ ID NO: 63 - protein, 7 aa, synthetic construct
  source 1..7: note = CDR
LVSKLDS

SEQ ID NO: 64 - protein, 9 aa, synthetic construct
  source 1..9: note = CDR
WQGSHFPQT

SEQ ID NO: 65 - protein, 115 aa, synthetic construct
  source 1..115: note = 0102 VH
EVQLVESGGGLVKPGGSLRLSCAASGFTFSTYAMSWVRQAPEKRLEWVATISDSDYYADNVKGRFTISRDNAKNSLYLQMNSLRAEDTAVYYCVRDDWDGDFDYWGQGTLVTVSS

SEQ ID NO: 66 - protein, 112 aa, synthetic construct
  source 1..112: note = 0102 VL
DVVMTQSPLSLPVTPGEPASISCKSTQSLLYSDGETYLNWLLQKPGQSPQRLIYLVSKLDSGVPDRFSGSGSGTDFTLKISRVEAEDVGVYYCWQGSHFPQTFGGGTKVEIK

SEQ ID NO: 67 - protein, 219 aa, synthetic construct
  source 1..219: note = Her HH13 LC
DIQMTQSPSSLSASVGDRVTITCRASQDVNTAVAWYQQKPGKAPKLLIYSASFLYSGVPSRFSGSRSGTDFTLTISSLQPEDFATYYCQQHYTTPPTFGQGTKVEIKRTVAAPSVFIFPPSDEQLKSGTASVVCLLNNFYPREAKVQWKVDNALQSGNSQESVTEQDSKDSTYSLSSTLTLSKADYEKHKVYACEVTHQGLSSPVTKSFNRGECGGGGY

SEQ ID NO: 68 - protein, 5 aa, synthetic construct
  source 1..5: note = CDR
DYAMH

SEQ ID NO: 69 - protein, 17 aa, synthetic construct
  source 1..17: note = CDR
AITWNSGHIDYADSVEG

SEQ ID NO: 70 - protein, 12 aa, synthetic construct
  source 1..12: note = CDR
VSYLSTASSLDY

SEQ ID NO: 71 - protein, 11 aa, synthetic construct
  source 1..11: note = CDR
RASQGIRNYLA

SEQ ID NO: 72 - protein, 7 aa, synthetic construct
  source 1..7: note = CDR
AASTLQS

SEQ ID NO: 73 - protein, 9 aa, synthetic construct
  source 1..9: note = CDR
QRYNRAPYT

SEQ ID NO: 74 - protein, 107 aa, synthetic construct
  source 1..107: note = TROP2 VH
EVQLVESGGGLVQPGRSLRLSCAASGFTFDDYAMHWVRQAPGKGLEWVSAITWNSGHIDYADSVEGRFTISRDNAKNSLYLQMNSLRAEDTAVYYCAKVSYLSTASS

SEQ ID NO: 75 - protein, 214 aa, synthetic construct; identical to SEQ ID NO: 43
  source 1..214: note = TROP2 VL

SEQ ID NO: 76 - protein, 5 aa, synthetic construct
  source 1..5: note = linker
YGGGG

SEQ ID NO: 77 - protein, 6 aa, synthetic construct
  source 1..6: note = linker
YGGGGS

SEQ ID NO: 78 - protein, 5 aa, synthetic construct
  source 1..5: note = linker
GGGGY

SEQ ID NO: 79 - protein, 6 aa, synthetic construct
  source 1..6: note = linker
SGGGGY

SEQ ID NO: 80 - protein, 14 aa, synthetic construct
  source 1..14: note = P-1
EQKLISEEDLGGSC

SEQ ID NO: 81 - protein, 10 aa, synthetic construct
  source 1..10: note = P-2
LRELHLNNNC

SEQ ID NO: 82 - protein, 98 aa, synthetic construct
  source 1..98: note = CH1 T135Y
ASTKGPSVFPLAPSSKSYSGGTAALGCLVKDYFPEPVTVSWNSGALTSGVHTFPAVLQSSGLYSLSSVVTVPSSSLGTQTYICNVNHKPSNTKVDKKV

SEQ ID NO: 83 - protein, 98 aa, synthetic construct
  source 1..98: note = CH1 G137Y
ASTKGPSVFPLAPSSKSTSYGTAALGCLVKDYFPEPVTVSWNSGALTSGVHTFPAVLQSSGLYSLSSVVTVPSSSLGTQTYICNVNHKPSNTKVDKKV

SEQ ID NO: 84 - protein, 98 aa, synthetic construct
  source 1..98: note = CH1 S192Y
ASTKGPSVFPLAPSSKSTSGGTAALGCLVKDYFPEPVTVSWNSGALTSGVHTFPAVLQSSGLYSLSSVVTVPSSYLGTQTYICNVNHKPSNTKVDKKV

SEQ ID NO: 85 - protein, 15 aa, synthetic construct
  source 1..15: note = T223Y
EPKSCDKYHTCPPCP

SEQ ID NO: 86 - protein, 110 aa, synthetic construct
  source 1..110: note = CH2 P329Y
APELLGGPSVFLFPPKPKDTLMISRTPEVTCVVVDVSHEDPEVKFNWYVDGVEVHNAKTKPREEQYNSTYRVVSVLTVLHQDWLNGKEYKCKVSNKALYAPIEKTISKAK

SEQ ID NO: 87 - protein, 107 aa, synthetic construct
  source 1..107: note = Ck S202Y
RTVAAPSVFIFPPSDEQLKSGTASVVCLLNNFYPREAKVQWKVDNALQSGNSQESVTEQDSKDSTYSLSSTLTLSKADYEKHKVYACEVTHQGLYSPVTKSFNRGEC

SEQ ID NO: 88 - protein, 98 aa, synthetic construct
  source 1..98: note = CH1 T135Y S192Y
ASTKGPSVFPLAPSSKSYSGGTAALGCLVKDYFPEPVTVSWNSGALTSGVHTFPAVLQSSGLYSLSSVVTVPSSYLGTQTYICNVNHKPSNTKVDKKV

SEQ ID NO: 89 - protein, 98 aa, synthetic construct
  source 1..98: note = CH1 G137Y S192Y
ASTKGPSVFPLAPSSKSTSYGTAALGCLVKDYFPEPVTVSWNSGALTSGVHTFPAVLQSSGLYSLSSVVTVPSSYLGTQTYICNVNHKPSNTKVDKKV

SEQ ID NO: 90 - protein, 98 aa, synthetic construct
  source 1..98: note = CH1 T135Y G137Y
ASTKGPSVFPLAPSSKSYSYGTAALGCLVKDYFPEPVTVSWNSGALTSGVHTFPAVLQSSGLYSLSSVVTVPSSSLGTQTYICNVNHKPSNTKVDKKV